European Patent Specification EP 3 468 988 B1, published January 31, 2024. Title: Peptides for the inhibition of parasite infections. Applicant: Aqua Health AS. The sequence listing filed with the application follows.

SEQUENCE LISTING (11 sequences)

SEQ ID NO: 1 - protein, 14 aa, Artificial
  Artificial peptide sequence
VPEPVVQSPITTTT

SEQ ID NO: 2 - protein, 20 aa, Artificial
  Artificial peptide sequence
VRCGRGRMLLLIERGQRFAT

SEQ ID NO: 3 - protein, 12 aa, Artificial
  Artificial peptide sequence
VLGEEWHMEGCM

SEQ ID NO: 4 - protein, 13 aa, Artificial
  Artificial peptide sequence
LMSFRKDAVMAIM

SEQ ID NO: 5 - protein, 10 aa, Artificial
  Artificial peptide sequence
KLTINDASLC

SEQ ID NO: 6 - protein, 17 aa, Artificial
  Artificial peptide sequence
TTTLLLHFTFDFNRVGV

SEQ ID NO: 7 - protein, 13 aa, Artificial
  Artificial peptide sequence
DVVQVGYQMDHII

SEQ ID NO: 8 - protein, 9 aa, Artificial
  Artificial peptide sequence
LNELETEMV

SEQ ID NO: 9 - protein, 13 aa, Artificial
  Artificial peptide sequence
LKFMLPRRWCTGC

SEQ ID NO: 10 - protein, 11 aa, Artificial
  Artificial peptide sequence
KFLHLDFNNGL

SEQ ID NO: 11 - protein, 17 aa, Artificial
  Aritificial peptide sequence
TPYYTTVNPTSPYTYDV